European Patent Application EP 4 458 460 A1, published November 6, 2024. Title: Method and Apparatus for producing peptide. Applicant: Yokogawa Electric Corporation. Application EP. The sequence listing filed with the application follows.

SEQUENCE LISTING (1 sequence)

SEQ ID NO: 1 - protein, 5 aa, synthetic construct
  REGION 1..5: note = Artificial peptide
EAEKL